European Patent Specification EP 3 417 052 B1, published February 15, 2023. Title: METHODS FOR EXPANDING AND DIFFERENTIATING B CELLS FOR PRODUCING ANTIBODY. Applicant: DUKE UNIVERSITY SUGA, Hiraku CANDANDO, Kathleen KOUNTIKOV, Evgueni KAMATA, Masahiro TEDDER, Thomas YOSHIZAKI, Ayumi MIYAGAKI, Tomomitsu. The sequence listing filed with the application follows.

SEQUENCE LISTING (70 sequences)

SEQ ID NO: 1 - DNA, 1090 bp, Artificial Sequence
  Synthetic: BLyS
taactctcctgaggggtgagccaagccctgccatgtagtgcacgcaggacatcaacaaacacagataacaggaaatgatccattccctgtggtcacttattctaaaggccccaaccttcaaagttcaagtagtgatatggatgactccacagaaagggagcagtcacgccttacttcttgccttaagaaaagagaagaaatgaaactgaaggagtgtgtttccatcctcccacggaaggaaagcccctctgtccgatcctccaaagacggaaagctgctggctgcaaccttgctgctggcactgctgtcttgctgcctcacggtggtgtctttctaccaggtggccgccctgcaaggggacctggccagcctccgggcagagctgcagggccaccacgcggagaagctgccagcaggagcaggagcccccaaggccggcctggaggaagctccagctgtcaccgcgggactgaaaatctttgaaccaccagctccaggagaaggcaactccagtcagaacagcagaaataagcgtgccgttcagggtccagaagaaacagtcactcaagactgcttgcaactgattgcagacagtgaaacaccaactatacaaaaaggatcttacacatttgttccatggcttctcagctttaaaaggggaagtgccctagaagaaaaagagaataaaatattggtcaaagaaactggttacttttttatatatggtcaggttttatatactgataagacctacgccatgggacatctaattcagaggaagaaggtccatgtctttggggatgaattgagtctggtgactttgtttcgatgtattcaaaatatgcctgaaacactacccaataattcctgctattcagctggcattgcaaaactggaagaaggagatgaactccaacttgcaataccaagagaaaatgcacaaatatcactggatggagatgtcacattttttggtgcattgaaactgctgtgacctacttacaccatgtctgtagctattttcctccctttctctgtacctctaagaagaaagaatctaactgaaaataccaaaaaaaaaaaaaaaaaa

SEQ ID NO: 2 - DNA, 1859 bp, Artificial Sequence
  Synthetic: CD154
actttgacagtcttctcatgctgcctctgccaccttctctgccagaagataccatttcaactttaacacagcatgatcgaaacatacaaccaaacttctccccgatctgcggccactggactgcccatcagcatgaaaatttttatgtatttacttactgtttttcttatcacccagatgattgggtcagcactttttgctgtgtatcttcatagaaggttggacaagatagaagatgaaaggaatcttcatgaagattttgtattcatgaaaacgatacagagatgcaacacaggagaaagatccttatccttactgaactgtgaggagattaaaagccagtttgaaggctttgtgaaggatataatgttaaacaaagaggagacgaagaaagaaaacagctttgaaatgcaaaaaggtgatcagaatcctcaaattgcggcacatgtcataagtgaggccagcagtaaaacaacatctgtgttacagtgggctgaaaaaggatactacaccatgagcaacaacttggtaaccctggaaaatgggaaacagctgaccgttaaaagacaaggactctattatatctatgcccaagtcaccttctgttccaatcgggaagcttcgagtcaagctccatttatagccagcctctgcctaaagtcccccggtagattcgagagaatcttactcagagctgcaaatacccacagttccgccaaaccttgcgggcaacaatccattcacttgggaggagtatttgaattgcaaccaggtgcttcggtgtttgtcaatgtgactgatccaagccaagtgagccatggcactggcttcacgtcctttggcttactcaaactctgaacagtgtcaccttgcaggctgtggtggagctgacgctgggagtcttcataatacagcacagcggttaagcccaccccctgttaactgcctatttataaccctaggatcctccttatggagaactatttattatacactccaaggcatgtagaactgtaataagtgaattacaggtcacatgaaaccaaaacgggccctgctccataagagcttatatatctgaagcagcaaccccactgatgcagacatccagagagtcctatgaaaagacaaggccattatgcacaggttgaattctgagtaaacagcagataacttgccaagttcagttttgtttctttgcgtgcagtgtctttccatggataatgcatttgatttatcagtgaagatgcagaagggaaatggggagcctcagctcacattcagttatggttgactctgggttcctatggccttgttggagggggccaggctctagaacgtctaacacagtggagaaccgaaaccccccccccccgccaccctctcggacagttattcattctctttcaatctctctctctccatctctctctttcagtctctctctctcaacctctttcttccaatctctctttctcaatctctctgtttccctttgtcagtctcttccctcccccagtctctcttctcaatccccctttctaacacacacacacacacacacacacacacacacacacacacacacacacacacagagtcaggccgttgctagtcagttctcttctttccaccctgtccctatctctaccactatagatgagggtgaggagtagggagtgcagccctgagcctgcccactcctcattacgaaatgactgtatttaaaggaaatctattgtatctacctgcagtctccattgtttccagagtgaacttgtaattatcttgttatttattttttgaataataaagacctcttaacattaagaaaaaaaaaaaaaaaaaaaaaaaaaaaa

SEQ ID NO: 3 - DNA, 870 bp, Artificial Sequence
  Synthetic: CD154
tctgccagaagataccatttcaactttaacacagcatgatcgaaacatacaaccaaacttctccccgatctgcggccactggactgcccatcagcatgaaaatttttatgtatttacttactgtttttcttatcacccagatgattgggtcagcactttttgctgtgtatcttcatagaaggttggacaagatagaagatgaaaggaatcttcatgaagattttgtattcatgaaaacgatacagagatgcaacacaggagaaagatccttatccttactgaactgtgaggagattaaaagccagtttgaaggctttgtgaaggatataatgttaaacaaagaggagacgaagaaagaaaacagctttgaaatgcaaaaaggtgatcagaatcctcaaattgcggcacatgtcataagtgaggccagcagtaaaacaacatctgtgttacagtgggctgaaaaaggatactacaccatgagcaacaacttggtaaccctggaaaatgggaaacagctgaccgttaaaagacaaggactctattatatctatgcccaagtcaccttctgttccaatcgggaagcttcgagtcaagctccatttatagccagcctctgcctaaagtcccccggtagattcgagagaatcttactcagagctgcaaatacccacagttccgccaaaccttgcgggcaacaatccattcacttgggaggagtatttgaattgcaaccaggtgcttcggtgtttgtcaatgtgactgatccaagccaagtgagccatggcactggcttcacgtcctttggcttactcaaactctgaacagtgtcaccttgcaggctgtggtggagctgacgctgggagtcttcat

SEQ ID NO: 4 - DNA, 564 bp, Artificial Sequence
  Synthetic: IL-21
ctgaagtgaaaacgagaccaaggtccagctctactgttggtacttatgagatccagtcctggcaacatggagaggattgtcatctgtctgatggtcatcttcttggggacactggtccacaaatcaagctcccaaggtcaagatcgccacatgattagaatgcgtcaacttatagatattgttgatcagctgaaaaattatgtgaatgacttggtccctgaatttctgccagctccagaagatgtagagacaaactgtgagtggtcagctttttcctgttttcagaaggcccaactaaagtcagcaaatacaggaaacaatgaaaggataatcaatgtatcaattaaaaagctgaagaggaaaccaccttccacaaatgcagggagaagacagaaacacagactaacatgcccttcatgtgattcttatgagaaaaaaccacccaaagaattcctagaaagattcaaatcacttctccaaaagatgattcatcagcatctgtcctctagaacacacggaagtgaagattcctgaggatctaacttgcagttggacattgttaca

SEQ ID NO: 5 - DNA, 20 bp, Artificial Sequence
  Synthetic: Reverse transcriptase (RT) primer  IgM
atggagtcgggaaggaagtc

SEQ ID NO: 6 - DNA, 19 bp, Artificial Sequence
  Synthetic: Reverse transcriptase (RT) primer  IgD
tcacggacgttgggtggta

SEQ ID NO: 7 - DNA, 19 bp, Artificial Sequence
  Synthetic: Reverse transcriptase (RT) primer  IgE
tcacggaggtggcattgga

SEQ ID NO: 8 - DNA, 19 bp, Artificial Sequence
  Synthetic: Reverse transcriptase (RT) primer  IgA1
caggcgatgaccacgttcc

SEQ ID NO: 9 - DNA, 19 bp, Artificial Sequence
  Synthetic: Reverse transcriptase (RT) primer  IgA2
catgcgacgaccacgttcc

SEQ ID NO: 10 - DNA, 20 bp, Artificial Sequence
  Synthetic: Reverse transcriptase (RT) primer  IgG
aggtgtgcacgccgctggtc

SEQ ID NO: 11 - DNA, 20 bp, Artificial Sequence
  Synthetic: Reverse transcriptase (RT) primer  IgKappa
gcaggcacacaacagaggca

SEQ ID NO: 12 - DNA, 17 bp, Artificial Sequence
  Synthetic: Reverse transcriptase (RT) primer  IgLambda
aggccactgtcacagct

SEQ ID NO: 13 - DNA, 24 bp, Artificial Sequence
  Synthetic: Forward Primer VH1-Internal
caggtgcagctggtrcagtctggg

SEQ ID NO: 14 - DNA, 26 bp, Artificial Sequence
  Synthetic: Forward Primer VH2-Internal
cagrgcaccttgarggagtctggtcc

SEQ ID NO: 15 - DNA, 24 bp, Artificial Sequence
  Synthetic: Forward Primer VH3-Internal
gaggtkcagctggtggagtctggg

SEQ ID NO: 16 - DNA, 22 bp, Artificial Sequence
  Synthetic: Forward Primer VH4-Internal
caggtgcagctgcaggagtcgg

SEQ ID NO: 17 - DNA, 25 bp, Artificial Sequence
  Synthetic: Forward Primer VH5-Internal
gargtgcagctggtgcagtctggag

SEQ ID NO: 18 - DNA, 26 bp, Artificial Sequence
  Synthetic: Forward Primer VH6-Internal
caggtacagctgcagcagtcaggtcc

SEQ ID NO: 19 - DNA, 22 bp, Artificial Sequence
  Synthetic: Forward Primer V-kappa-1-Internal
gacatccagwtgacccagtctc

SEQ ID NO: 20 - DNA, 25 bp, Artificial Sequence
  Synthetic: Forward Primer V-kappa-2-Internal
gatattgtgatgacccagwctccac

SEQ ID NO: 21 - DNA, 24 bp, Artificial Sequence
  Synthetic: Forward Primer V-kappa-3-Internal
gaaattgtgttgacrcagtctcca

SEQ ID NO: 22 - DNA, 22 bp, Artificial Sequence
  Synthetic: Forward Primer V-kappa-4-Internal
gacatcgtgatgacccagtctc

SEQ ID NO: 23 - DNA, 22 bp, Artificial Sequence
  Synthetic: Forward Primer V-kappa-5-Internal
gaaacgacactcacgcagtctc

SEQ ID NO: 24 - DNA, 24 bp, Artificial Sequence
  Synthetic: Forward Primer V-kappa-6-Internal
gaaattgtgctgacwcagtctcca

SEQ ID NO: 25 - DNA, 21 bp, Artificial Sequence
  Synthetic: Forward Primer V-kappa-7-Internal
gacattgtgctgacccagtct

SEQ ID NO: 26 - DNA, 20 bp, Artificial Sequence
  Synthetic: Forward Primer V-lambda-1-Internal
cagtctgtgytgackcagcc

SEQ ID NO: 27 - DNA, 20 bp, Artificial Sequence
  Synthetic: Forward Primer V-lambda-2-Internal
cagtctgccctgactcagcc

SEQ ID NO: 28 - DNA, 22 bp, Artificial Sequence
  Synthetic: Forward Primer V-lambda-3-Internal
tcytatgagctgacwcagccac

SEQ ID NO: 29 - DNA, 23 bp, Artificial Sequence
  Synthetic: Forward Primer V-lambda-31-Internal
tcttctgagctgactcaggaccc

SEQ ID NO: 30 - DNA, 20 bp, Artificial Sequence
  Synthetic: Forward Primer V-lambda-4ab-Internal
cagcytgtgctgactcaatc

SEQ ID NO: 31 - DNA, 19 bp, Artificial Sequence
  Synthetic: Forward Primer V-lambda-4c-Internal
ctgcctgtgctgactcagc

SEQ ID NO: 32 - DNA, 20 bp, Artificial Sequence
  Synthetic: Forward Primer V-lambda-5/9-Internal
cagsctgtgctgactcagcc

SEQ ID NO: 33 - DNA, 25 bp, Artificial Sequence
  Synthetic: Forward Primer V-lambda-6-Internal
aattttatgctgactcagccccact

SEQ ID NO: 34 - DNA, 21 bp, Artificial Sequence
  Synthetic: Forward Primer V-lambda-7/8-Internal
cagrctgtggtgacycaggag

SEQ ID NO: 35 - DNA, 18 bp, Artificial Sequence
  Synthetic: Forward Primer V-lambda-10-Internal
caggcagggcwgactcag

SEQ ID NO: 36 - DNA, 21 bp, Artificial Sequence
  Synthetic: Reverse Primer IgA-1-Internal
gctggtgctgcagaggctcag

SEQ ID NO: 37 - DNA, 21 bp, Artificial Sequence
  Synthetic: Reverse Primer IgA-2-Internal
gctggtgctgtcgaggctcag

SEQ ID NO: 38 - DNA, 23 bp, Artificial Sequence
  Synthetic: Reverse Primer IgD-Internal
gtgtctgcaccctgatatgatgg

SEQ ID NO: 39 - DNA, 9 bp, Artificial Sequence
  Synthetic: Reverse Primer IgG-Internal
gctcytgga

SEQ ID NO: 40 - DNA, 22 bp, Artificial Sequence
  Synthetic: Reverse Primer IgM-Internal
ggaattctcacaggagacgagg

SEQ ID NO: 41 - DNA, 21 bp, Artificial Sequence
  Synthetic: Reverse Primer C-kappa- Internal
gggaagatgaagacagatggt

SEQ ID NO: 42 - DNA, 20 bp, Artificial Sequence
  Synthetic: Forward Primer VH1-External
ccatggactggacctggagg

SEQ ID NO: 43 - DNA, 19 bp, Artificial Sequence
  Synthetic: Forward Primer VH2-External
atggacatactttgttcca

SEQ ID NO: 44 - DNA, 20 bp, Artificial Sequence
  Synthetic: Forward Primer VH3-External
ccatggagtttgggctgagc

SEQ ID NO: 45 - DNA, 20 bp, Artificial Sequence
  Synthetic: Forward Primer VH4-External
atgaaacacctgtggttctt

SEQ ID NO: 46 - DNA, 20 bp, Artificial Sequence
  Synthetic: Forward Primer VH5-External
atggggtcaaccgccatcct

SEQ ID NO: 47 - DNA, 20 bp, Artificial Sequence
  Synthetic: Forward Primer VH6-External
atgtctgtctccttcctcat

SEQ ID NO: 48 - DNA, 17 bp, Artificial Sequence
  Synthetic: Forward Primer V-kappa-1/2-External
gctcagctcctggggct

SEQ ID NO: 49 - DNA, 17 bp, Artificial Sequence
  Synthetic: Forward Primer V-kappa-3-External
ggaarccccagcdcagc

SEQ ID NO: 50 - DNA, 19 bp, Artificial Sequence
  Synthetic: Forward Primer V-kappa-4/5-External
ctsttsctytggatctctg

SEQ ID NO: 51 - DNA, 17 bp, Artificial Sequence
  Synthetic: Forward Primer V-kappa-6/7-External
ctsctgctctgggytcc

SEQ ID NO: 52 - DNA, 17 bp, Artificial Sequence
  Synthetic: Forward Primer V-lambda-1-External
cctgggcccagtctgtg

SEQ ID NO: 53 - DNA, 18 bp, Artificial Sequence
  Synthetic: Forward Primer V-lambda-2-External
ctcctcasyctcctcact

SEQ ID NO: 54 - DNA, 18 bp, Artificial Sequence
  Synthetic: Forward Primer V-lambda-3-External
ggcctcctatgwgctgac

SEQ ID NO: 55 - DNA, 23 bp, Artificial Sequence
  Synthetic: Forward Primer V-lambda-31-External
gttctgtggtttcttctgagctg

SEQ ID NO: 56 - DNA, 18 bp, Artificial Sequence
  Synthetic: Forward Primer V-lambda-4ab-External
acagggtctctctcccag

SEQ ID NO: 57 - DNA, 19 bp, Artificial Sequence
  Synthetic: Forward Primer V-lambda-4c-External
acaggtctctgtgctctgc

SEQ ID NO: 58 - DNA, 17 bp, Artificial Sequence
  Synthetic: Forward Primer V-lambda-5/9-External
ccctctcscagsctgtg

SEQ ID NO: 59 - DNA, 19 bp, Artificial Sequence
  Synthetic: Forward Primer V-lambda-6-External
tcttgggccaattttatgc

SEQ ID NO: 60 - DNA, 19 bp, Artificial Sequence
  Synthetic: Forward Primer V-lambda-7/8-External
attcycagrctgtggtgac

SEQ ID NO: 61 - DNA, 17 bp, Artificial Sequence
  Synthetic: Forward Primer V-lambda-10-External
cagtggtccaggcaggg

SEQ ID NO: 62 - DNA, 20 bp, Artificial Sequence
  Synthetic: Reverse Primer IgA-1-External
cgaygaccacgttcccatct

SEQ ID NO: 63 - DNA, 24 bp, Artificial Sequence
  Synthetic: Reverse Primer IgD-External
ctgttatcctttgggtgtctgcac

SEQ ID NO: 64 - DNA, 20 bp, Artificial Sequence
  Synthetic: Reverse Primer IgG-External
cgcctgagttccacgacacc

SEQ ID NO: 65 - DNA, 20 bp, Artificial Sequence
  Synthetic: Reverse Primer IgM-External
ccgacggggaattctcacag

SEQ ID NO: 66 - DNA, 20 bp, Artificial Sequence
  Synthetic: Reverse Primer C-kappa- External
gaggcagttccagatttcaa

SEQ ID NO: 67 - DNA, 17 bp, Artificial Sequence
  Synthetic: Reverse Primer C-lambda- External
aggccactgtcacagct

SEQ ID NO: 68 - protein, 261 aa, Artificial Sequence
  Synthetic: CD154 polypeptide sequence
MIETYNQTSPRSAATGLPISMKIFMYLLTVFLITQMIGSALFAVYLHRRLDKIEDERNLHEDFVFMKTIQRCNTGERSLSLLNCEEIKSQFEGFVKDIMLNKEETKKENSFEMQKGDQNPQIAAHVISEASSKTTSVLQWAEKGYYTMSNNLVTLENGKQLTVKRQGLYYIYAQVTFCSNREASSQAPFIASLCLKSPGRFERILLRAANTHSSAKPCGQQSIHLGGVFELQPGASVFVNVTDPSQVSHGTGFTSFGLLKL

SEQ ID NO: 69 - protein, 285 aa, Artificial Sequence
  Synthetic: BLyS polypeptide sequence
MDDSTEREQSRLTSCLKKREEMKLKECVSILPRKESPSVRSSKDGKLLAATLLLALLSCCLTVVSFYQVAALQGDLASLRAELQGHHAEKLPAGAGAPKAGLEEAPAVTAGLKIFEPPAPGEGNSSQNSRNKRAVQGPEETVTQDCLQLIADSETPTIQKGSYTFVPWLLSFKRGSALEEKENKILVKETGYFFIYGQVLYTDKTYAMGHLIQRKKVHVFGDELSLVTLFRCIQNMPETLPNNSCYSAGIAKLEEGDELQLAIPRENAQISLDGDVTFFGALKLL

SEQ ID NO: 70 - protein, 162 aa, Artificial Sequence
  Synthetic: IL-21 polypeptide sequence
MRSSPGNMERIVICLMVIFLGTLVHKSSSQGQDRHMIRMRQLIDIVDQLKNYVNDLVPEFLPAPEDVETNCEWSAFSCFQKAQLKSANTGNNERIINVSIKKLKRKPPSTNAGRRQKHRLTCPSCDSYEKKPPKEFLERFKSLLQKMIHQHLSSRTHGSEDS